European Patent Specification EP 3 559 030 B1, published April 3, 2024. Title: ANTI-IL-5 ANTIBODIES. Applicant: CEPHALON, INC. The sequence listing filed with the application follows.

SEQUENCE LISTING (75 sequences)

SEQ ID NO: 1 - protein, 11 aa, Artificial Sequence
  Description of Artificial Sequence: Synthetic peptide
  MOD_RES (2)..(2): Gly or Lys
  MOD_RES (3)..(3): Asn or Asp
  MOD_RES (4)..(4): Asn or His
  MOD_RES (5)..(5): Ile or Ala
  MOD_RES (6)..(6): Gly or Asp
  MOD_RES (7)..(7): Ser or Lys
  MOD_RES (9)..(9): Asn or His
  MOD_RES (10)..(10): Val or Ala
GXXXXXXKXXY

SEQ ID NO: 2 - protein, 7 aa, Artificial Sequence
  Description of Artificial Sequence: Synthetic peptide
  MOD_RES (3)..(3): Ser or Leu
  MOD_RES (4)..(4): Asp or Ser
DDXXRPS

SEQ ID NO: 3 - protein, 11 aa, Artificial Sequence
  Description of Artificial Sequence: Synthetic peptide
  MOD_RES (4)..(4): Asp or Leu
  MOD_RES (9)..(9): His, Ser, Tyr or Asp
  MOD_RES (11)..(11): Val, Ala or Trp
QVWXSSSDXVX

SEQ ID NO: 4 - protein, 12 aa, Artificial Sequence
  Description of Artificial Sequence: Synthetic peptide
GGSISNGGYYWS

SEQ ID NO: 5 - protein, 11 aa, Artificial Sequence
  Description of Artificial Sequence: Synthetic peptide
GGNNIGSKNVY

SEQ ID NO: 6 - protein, 9 aa, Artificial Sequence
  Description of Artificial Sequence: Synthetic peptide
YIYYSGSTY

SEQ ID NO: 7 - protein, 7 aa, Artificial Sequence
  Description of Artificial Sequence: Synthetic peptide
DDSDRPS

SEQ ID NO: 8 - protein, 7 aa, Artificial Sequence
  Description of Artificial Sequence: Synthetic peptide
LGNWFDY

SEQ ID NO: 9 - protein, 11 aa, Artificial Sequence
  Description of Artificial Sequence: Synthetic peptide
QVWYSSSDHVV

SEQ ID NO: 10 - protein, 117 aa, Artificial Sequence
  Description of Artificial Sequence: Synthetic polypeptide
QVQLQESGPGLVKPSQTLSLTCTVSGGSISNGGYYWSWIRQHPGKGLEWIGYIYYSGSTYYNPSLKSRVSISVDTSKNQFSLKLNSVTAADTAVYYCASLGNWFDYWGQGTLVTVSS

SEQ ID NO: 11 - protein, 109 aa, Artificial Sequence
  Description of Artificial Sequence: Synthetic polypeptide
SSILTQPPSVSVAPGQTARITCGGNNIGSKNVYWYQQKPGQAPVLVVHDDSDRPSGIPERFSGSNSGNTATLTISRVEVGDEADYSCQVWYSSSDHVVFGGGTKLTVLG

SEQ ID NO: 12 - protein, 446 aa, Artificial Sequence
  Description of Artificial Sequence: Synthetic polypeptide
QVQLQESGPGLVKPSQTLSLTCTVSGGSISNGGYYWSWIRQHPGKGLEWIGYIYYSGSTYYNPSLKSRVSISVDTSKNQFSLKLNSVTAADTAVYYCASLGNWFDYWGQGTLVTVSSASTKGPSVFPLAPSSKSTSGGTAALGCLVKDYFPEPVTVSWNSGALTSGVHTFPAVLQSSGLYSLSSVVTVPSSSLGTQTYICNVNHKPSNTKVDKKVEPKSCDKTHTCPPCPAPELLGGPSVFLFPPKPKDTLMISRTPEVTCVVVDVSHEDPEVKFNWYVDGVEVHNAKTKPREEQYNSTYRVVSVLTVLHQDWLNGKEYKCKVSNKALPAPIEKTISKAKGQPREPQVYTLPPSRDELTKNQVSLTCLVKGFYPSDIAVEWESNGQPENNYKTTPPVLDSDGSFFLYSKLTVDKSRWQQGNVFSCSVMHEALHNHYTQKSLSLSPG

SEQ ID NO: 13 - protein, 214 aa, Artificial Sequence
  Description of Artificial Sequence: Synthetic polypeptide
SSILTQPPSVSVAPGQTARITCGGNNIGSKNVYWYQQKPGQAPVLVVHDDSDRPSGIPERFSGSNSGNTATLTISRVEVGDEADYSCQVWYSSSDHVVFGGGTKLTVLGQPKAAPSVTLFPPSSEELQANKATLVCLISDFYPGAVTVAWKADSSPVKAGVETTTPSKQSNNKYAASSYLSLTPEQWKSHRSYSCQVTHEGSTVEKTVAPTECS

SEQ ID NO: 14 - protein, 443 aa, Artificial Sequence
  Description of Artificial Sequence: Synthetic polypeptide
QVQLQESGPGLVKPSQTLSLTCTVSGGSISNGGYYWSWIRQHPGKGLEWIGYIYYSGSTYYNPSLKSRVSISVDTSKNQFSLKLNSVTAADTAVYYCASLGNWFDYWGQGTLVTVSSASTKGPSVFPLAPCSRSTSESTAALGCLVKDYFPEPVTVSWNSGALTSGVHTFPAVLQSSGLYSLSSVVTVPSSSLGTKTYTCNVDHKPSNTKVDKRVESKYGPPCPPCPAPEFLGGPSVFLFPPKPKDTLMISRTPEVTCVVVDVSQEDPEVQFNWYVDGVEVHNAKTKPREEQFNSTYRVVSVLTVLHQDWLNGKEYKCKVSNKGLPSSIEKTISKAKGQPREPQVYTLPPSQEEMTKNQVSLTCLVKGFYPSDIAVEWESNGQPENNYKTTPPVLDSDGSFFLYSRLTVDKSRWQEGNVFSCSVMHEALHNHYTQKSLSLSLG

SEQ ID NO: 15 - protein, 11 aa, Artificial Sequence
  Description of Artificial Sequence: Synthetic peptide
QVWDSSSDHVV

SEQ ID NO: 16 - protein, 117 aa, Artificial Sequence
  Description of Artificial Sequence: Synthetic polypeptide
QVQLQESGPGLVKPSQTLSLTCTVSGGSISNGGYYWSWIRQHPGKGLEWIGYIYYSGSTYYNPSLKSRVTISVDTSKNQFSLKLSSVTAADTAVYYCASLGNWFDYWGQGTLVTVSS

SEQ ID NO: 17 - protein, 109 aa, Artificial Sequence
  Description of Artificial Sequence: Synthetic polypeptide
SYVLTQPPSVSVAPGQTARITCGGNNIGSKNVYWYQQKPGQAPVLVVHDDSDRPSGIPERFSGSNSGNTATLTISRVEVGDEADYSCQVWDSSSDHVVFGGGTKLTVLG

SEQ ID NO: 18 - protein, 443 aa, Artificial Sequence
  Description of Artificial Sequence: Synthetic polypeptide
QVQLQESGPGLVKPSQTLSLTCTVSGGSISNGGYYWSWIRQHPGKGLEWIGYIYYSGSTYYNPSLKSRVTISVDTSKNQFSLKLSSVTAADTAVYYCASLGNWFDYWGQGTLVTVSSASTKGPSVFPLAPCSRSTSESTAALGCLVKDYFPEPVTVSWNSGALTSGVHTFPAVLQSSGLYSLSSVVTVPSSSLGTKTYTCNVDHKPSNTKVDKRVESKYGPPCPPCPAPEFLGGPSVFLFPPKPKDTLMISRTPEVTCVVVDVSQEDPEVQFNWYVDGVEVHNAKTKPREEQFNSTYRVVSVLTVLHQDWLNGKEYKCKVSNKGLPSSIEKTISKAKGQPREPQVYTLPPSQEEMTKNQVSLTCLVKGFYPSDIAVEWESNGQPENNYKTTPPVLDSDGSFFLYSRLTVDKSRWQEGNVFSCSVMHEALHNHYTQKSLSLSLG

SEQ ID NO: 19 - protein, 214 aa, Artificial Sequence
  Description of Artificial Sequence: Synthetic polypeptide
SYVLTQPPSVSVAPGQTARITCGGNNIGSKNVYWYQQKPGQAPVLVVHDDSDRPSGIPERFSGSNSGNTATLTISRVEVGDEADYSCQVWDSSSDHVVFGGGTKLTVLGQPKAAPSVTLFPPSSEELQANKATLVCLISDFYPGAVTVAWKADSSPVKAGVETTTPSKQSNNKYAASSYLSLTPEQWKSHRSYSCQVTHEGSTVEKTVAPTECS

SEQ ID NO: 20 - protein, 443 aa, Artificial Sequence
  Description of Artificial Sequence: Synthetic polypeptide
QVQLQESGPGLVKPSQTLSLTCTVSGGSISNGGYYWSWIRQHPGKGLEWIGYIYYSGSTYYNPSLKSRVTISVDTSKNQFSLKLSSVTAADTAVYYCASLGNWFDYWGQGTLVTVSSASTKGPSVFPLAPCSRSTSESTAALGCLVKDYFPEPVTVSWNSGALTSGVHTFPAVLQSSGLYSLSSVVTVPSSSLGTKTYTCNVDHKPSNTKVDKRVESKYGPPCPPCPAPEFLGGPSVFLFPPKPKDTLYITREPEVTCVVVDVSQEDPEVQFNWYVDGVEVHNAKTKPREEQFNSTYRVVSVLTVLHQDWLNGKEYKCKVSNKGLPSSIEKTISKAKGQPREPQVYTLPPSQEEMTKNQVSLTCLVKGFYPSDIAVEWESNGQPENNYKTTPPVLDSDGSFFLYSRLTVDKSRWQEGNVFSCSVMHEALHNHYTQKSLSLSLG

SEQ ID NO: 21 - protein, 11 aa, Artificial Sequence
  Description of Artificial Sequence: Synthetic peptide
GKNNIGSKNVY

SEQ ID NO: 22 - protein, 109 aa, Artificial Sequence
  Description of Artificial Sequence: Synthetic polypeptide
SYVLTQPPSVSVAPGQTARITCGKNNIGSKNVYWYQQKPGQAPVLVVHDDSDRPSGIPERFSGSNSGNTATLTISRVEVGDEADYSCQVWDSSSDHVVFGGGTKLTVLG

SEQ ID NO: 23 - protein, 214 aa, Artificial Sequence
  Description of Artificial Sequence: Synthetic polypeptide
SYVLTQPPSVSVAPGQTARITCGKNNIGSKNVYWYQQKPGQAPVLVVHDDSDRPSGIPERFSGSNSGNTATLTISRVEVGDEADYSCQVWDSSSDHVVFGGGTKLTVLGQPKAAPSVTLFPPSSEELQANKATLVCLISDFYPGAVTVAWKADSSPVKAGVETTTPSKQSNNKYAASSYLSLTPEQWKSHRSYSCQVTHEGSTVEKTVAPTECS

SEQ ID NO: 24 - protein, 11 aa, Artificial Sequence
  Description of Artificial Sequence: Synthetic peptide
GGDNIGSKNVY

SEQ ID NO: 25 - protein, 109 aa, Artificial Sequence
  Description of Artificial Sequence: Synthetic polypeptide
SYVLTQPPSVSVAPGQTARITCGGDNIGSKNVYWYQQKPGQAPVLVVHDDSDRPSGIPERFSGSNSGNTATLTISRVEVGDEADYSCQVWDSSSDHVVFGGGTKLTVLG

SEQ ID NO: 26 - protein, 214 aa, Artificial Sequence
  Description of Artificial Sequence: Synthetic polypeptide
SYVLTQPPSVSVAPGQTARITCGGDNIGSKNVYWYQQKPGQAPVLVVHDDSDRPSGIPERFSGSNSGNTATLTISRVEVGDEADYSCQVWDSSSDHVVFGGGTKLTVLGQPKAAPSVTLFPPSSEELQANKATLVCLISDFYPGAVTVAWKADSSPVKAGVETTTPSKQSNNKYAASSYLSLTPEQWKSHRSYSCQVTHEGSTVEKTVAPTECS

SEQ ID NO: 27 - protein, 11 aa, Artificial Sequence
  Description of Artificial Sequence: Synthetic peptide
GGNHIGSKNVY

SEQ ID NO: 28 - protein, 109 aa, Artificial Sequence
  Description of Artificial Sequence: Synthetic polypeptide
SYVLTQPPSVSVAPGQTARITCGGNHIGSKNVYWYQQKPGQAPVLVVHDDSDRPSGIPERFSGSNSGNTATLTISRVEVGDEADYSCQVWDSSSDHVVFGGGTKLTVLG

SEQ ID NO: 29 - protein, 214 aa, Artificial Sequence
  Description of Artificial Sequence: Synthetic polypeptide
SYVLTQPPSVSVAPGQTARITCGGNHIGSKNVYWYQQKPGQAPVLVVHDDSDRPSGIPERFSGSNSGNTATLTISRVEVGDEADYSCQVWDSSSDHVVFGGGTKLTVLGQPKAAPSVTLFPPSSEELQANKATLVCLISDFYPGAVTVAWKADSSPVKAGVETTTPSKQSNNKYAASSYLSLTPEQWKSHRSYSCQVTHEGSTVEKTVAPTECS

SEQ ID NO: 30 - protein, 11 aa, Artificial Sequence
  Description of Artificial Sequence: Synthetic peptide
GGNNAGSKNVY

SEQ ID NO: 31 - protein, 109 aa, Artificial Sequence
  Description of Artificial Sequence: Synthetic polypeptide
SYVLTQPPSVSVAPGQTARITCGGNNAGSKNVYWYQQKPGQAPVLVVHDDSDRPSGIPERFSGSNSGNTATLTISRVEVGDEADYSCQVWDSSSDHVVFGGGTKLTVLG

SEQ ID NO: 32 - protein, 214 aa, Artificial Sequence
  Description of Artificial Sequence: Synthetic polypeptide
SYVLTQPPSVSVAPGQTARITCGGNNAGSKNVYWYQQKPGQAPVLVVHDDSDRPSGIPERFSGSNSGNTATLTISRVEVGDEADYSCQVWDSSSDHVVFGGGTKLTVLGQPKAAPSVTLFPPSSEELQANKATLVCLISDFYPGAVTVAWKADSSPVKAGVETTTPSKQSNNKYAASSYLSLTPEQWKSHRSYSCQVTHEGSTVEKTVAPTECS

SEQ ID NO: 33 - protein, 11 aa, Artificial Sequence
  Description of Artificial Sequence: Synthetic peptide
GGNNIGKKNVY

SEQ ID NO: 34 - protein, 109 aa, Artificial Sequence
  Description of Artificial Sequence: Synthetic polypeptide
SYVLTQPPSVSVAPGQTARITCGGNNIGKKNVYWYQQKPGQAPVLVVHDDSDRPSGIPERFSGSNSGNTATLTISRVEVGDEADYSCQVWDSSSDHVVFGGGTKLTVLG

SEQ ID NO: 35 - protein, 214 aa, Artificial Sequence
  Description of Artificial Sequence: Synthetic polypeptide
SYVLTQPPSVSVAPGQTARITCGGNNIGKKNVYWYQQKPGQAPVLVVHDDSDRPSGIPERFSGSNSGNTATLTISRVEVGDEADYSCQVWDSSSDHVVFGGGTKLTVLGQPKAAPSVTLFPPSSEELQANKATLVCLISDFYPGAVTVAWKADSSPVKAGVETTTPSKQSNNKYAASSYLSLTPEQWKSHRSYSCQVTHEGSTVEKTVAPTECS

SEQ ID NO: 36 - protein, 11 aa, Artificial Sequence
  Description of Artificial Sequence: Synthetic peptide
GGNNIGSKHVY

SEQ ID NO: 37 - protein, 109 aa, Artificial Sequence
  Description of Artificial Sequence: Synthetic polypeptide
SYVLTQPPSVSVAPGQTARITCGGNNIGSKHVYWYQQKPGQAPVLVVHDDSDRPSGIPERFSGSNSGNTATLTISRVEVGDEADYSCQVWDSSSDHVVFGGGTKLTVLG

SEQ ID NO: 38 - protein, 214 aa, Artificial Sequence
  Description of Artificial Sequence: Synthetic polypeptide
SYVLTQPPSVSVAPGQTARITCGGNNIGSKHVYWYQQKPGQAPVLVVHDDSDRPSGIPERFSGSNSGNTATLTISRVEVGDEADYSCQVWDSSSDHVVFGGGTKLTVLGQPKAAPSVTLFPPSSEELQANKATLVCLISDFYPGAVTVAWKADSSPVKAGVETTTPSKQSNNKYAASSYLSLTPEQWKSHRSYSCQVTHEGSTVEKTVAPTECS

SEQ ID NO: 39 - protein, 11 aa, Artificial Sequence
  Description of Artificial Sequence: Synthetic peptide
GGNNIGSKNAY

SEQ ID NO: 40 - protein, 109 aa, Artificial Sequence
  Description of Artificial Sequence: Synthetic polypeptide
SYVLTQPPSVSVAPGQTARITCGGNNIGSKNAYWYQQKPGQAPVLVVHDDSDRPSGIPERFSGSNSGNTATLTISRVEVGDEADYSCQVWDSSSDHVVFGGGTKLTVLG

SEQ ID NO: 41 - protein, 214 aa, Artificial Sequence
  Description of Artificial Sequence: Synthetic polypeptide
SYVLTQPPSVSVAPGQTARITCGGNNIGSKNAYWYQQKPGQAPVLVVHDDSDRPSGIPERFSGSNSGNTATLTISRVEVGDEADYSCQVWDSSSDHVVFGGGTKLTVLGQPKAAPSVTLFPPSSEELQANKATLVCLISDFYPGAVTVAWKADSSPVKAGVETTTPSKQSNNKYAASSYLSLTPEQWKSHRSYSCQVTHEGSTVEKTVAPTECS

SEQ ID NO: 42 - protein, 7 aa, Artificial Sequence
  Description of Artificial Sequence: Synthetic peptide
DDLDRPS

SEQ ID NO: 43 - protein, 109 aa, Artificial Sequence
  Description of Artificial Sequence: Synthetic polypeptide
SYVLTQPPSVSVAPGQTARITCGGNNIGSKNVYWYQQKPGQAPVLVVHDDLDRPSGIPERFSGSNSGNTATLTISRVEVGDEADYSCQVWDSSSDHVVFGGGTKLTVLG

SEQ ID NO: 44 - protein, 214 aa, Artificial Sequence
  Description of Artificial Sequence: Synthetic polypeptide
SYVLTQPPSVSVAPGQTARITCGGNNIGSKNVYWYQQKPGQAPVLVVHDDLDRPSGIPERFSGSNSGNTATLTISRVEVGDEADYSCQVWDSSSDHVVFGGGTKLTVLGQPKAAPSVTLFPPSSEELQANKATLVCLISDFYPGAVTVAWKADSSPVKAGVETTTPSKQSNNKYAASSYLSLTPEQWKSHRSYSCQVTHEGSTVEKTVAPTECS

SEQ ID NO: 45 - protein, 7 aa, Artificial Sequence
  Description of Artificial Sequence: Synthetic peptide
DDSSRPS

SEQ ID NO: 46 - protein, 109 aa, Artificial Sequence
  Description of Artificial Sequence: Synthetic polypeptide
SYVLTQPPSVSVAPGQTARITCGGNNIGSKNVYWYQQKPGQAPVLVVHDDSSRPSGIPERFSGSNSGNTATLTISRVEVGDEADYSCQVWDSSSDHVVFGGGTKLTVLG

SEQ ID NO: 47 - protein, 214 aa, Artificial Sequence
  Description of Artificial Sequence: Synthetic polypeptide
SYVLTQPPSVSVAPGQTARITCGGNNIGSKNVYWYQQKPGQAPVLVVHDDSSRPSGIPERFSGSNSGNTATLTISRVEVGDEADYSCQVWDSSSDHVVFGGGTKLTVLGQPKAAPSVTLFPPSSEELQANKATLVCLISDFYPGAVTVAWKADSSPVKAGVETTTPSKQSNNKYAASSYLSLTPEQWKSHRSYSCQVTHEGSTVEKTVAPTECS

SEQ ID NO: 48 - protein, 11 aa, Artificial Sequence
  Description of Artificial Sequence: Synthetic peptide
QVWLSSSDHVV

SEQ ID NO: 49 - protein, 109 aa, Artificial Sequence
  Description of Artificial Sequence: Synthetic polypeptide
SYVLTQPPSVSVAPGQTARITCGGNNIGSKNVYWYQQKPGQAPVLVVHDDSDRPSGIPERFSGSNSGNTATLTISRVEVGDEADYSCQVWLSSSDHVVFGGGTKLTVLG

SEQ ID NO: 50 - protein, 214 aa, Artificial Sequence
  Description of Artificial Sequence: Synthetic polypeptide
SYVLTQPPSVSVAPGQTARITCGGNNIGSKNVYWYQQKPGQAPVLVVHDDSDRPSGIPERFSGSNSGNTATLTISRVEVGDEADYSCQVWLSSSDHVVFGGGTKLTVLGQPKAAPSVTLFPPSSEELQANKATLVCLISDFYPGAVTVAWKADSSPVKAGVETTTPSKQSNNKYAASSYLSLTPEQWKSHRSYSCQVTHEGSTVEKTVAPTECS

SEQ ID NO: 51 - protein, 11 aa, Artificial Sequence
  Description of Artificial Sequence: Synthetic peptide
QVWDSSSDSVV

SEQ ID NO: 52 - protein, 109 aa, Artificial Sequence
  Description of Artificial Sequence: Synthetic polypeptide
SYVLTQPPSVSVAPGQTARITCGGNNIGSKNVYWYQQKPGQAPVLVVHDDSDRPSGIPERFSGSNSGNTATLTISRVEVGDEADYSCQVWDSSSDSVVFGGGTKLTVLG

SEQ ID NO: 53 - protein, 214 aa, Artificial Sequence
  Description of Artificial Sequence: Synthetic polypeptide
SYVLTQPPSVSVAPGQTARITCGGNNIGSKNVYWYQQKPGQAPVLVVHDDSDRPSGIPERFSGSNSGNTATLTISRVEVGDEADYSCQVWDSSSDSVVFGGGTKLTVLGQPKAAPSVTLFPPSSEELQANKATLVCLISDFYPGAVTVAWKADSSPVKAGVETTTPSKQSNNKYAASSYLSLTPEQWKSHRSYSCQVTHEGSTVEKTVAPTECS

SEQ ID NO: 54 - protein, 11 aa, Artificial Sequence
  Description of Artificial Sequence: Synthetic peptide
QVWDSSSDYVV

SEQ ID NO: 55 - protein, 109 aa, Artificial Sequence
  Description of Artificial Sequence: Synthetic polypeptide
SYVLTQPPSVSVAPGQTARITCGGNNIGSKNVYWYQQKPGQAPVLVVHDDSDRPSGIPERFSGSNSGNTATLTISRVEVGDEADYSCQVWDSSSDYVVFGGGTKLTVLG

SEQ ID NO: 56 - protein, 214 aa, Artificial Sequence
  Description of Artificial Sequence: Synthetic polypeptide
SYVLTQPPSVSVAPGQTARITCGGNNIGSKNVYWYQQKPGQAPVLVVHDDSDRPSGIPERFSGSNSGNTATLTISRVEVGDEADYSCQVWDSSSDYVVFGGGTKLTVLGQPKAAPSVTLFPPSSEELQANKATLVCLISDFYPGAVTVAWKADSSPVKAGVETTTPSKQSNNKYAASSYLSLTPEQWKSHRSYSCQVTHEGSTVEKTVAPTECS

SEQ ID NO: 57 - protein, 11 aa, Artificial Sequence
  Description of Artificial Sequence: Synthetic peptide
QVWDSSSDDVV

SEQ ID NO: 58 - protein, 109 aa, Artificial Sequence
  Description of Artificial Sequence: Synthetic polypeptide
SYVLTQPPSVSVAPGQTARITCGGNNIGSKNVYWYQQKPGQAPVLVVHDDSDRPSGIPERFSGSNSGNTATLTISRVEVGDEADYSCQVWDSSSDDVVFGGGTKLTVLG

SEQ ID NO: 59 - protein, 214 aa, Artificial Sequence
  Description of Artificial Sequence: Synthetic polypeptide
SYVLTQPPSVSVAPGQTARITCGGNNIGSKNVYWYQQKPGQAPVLVVHDDSDRPSGIPERFSGSNSGNTATLTISRVEVGDEADYSCQVWDSSSDDVVFGGGTKLTVLGQPKAAPSVTLFPPSSEELQANKATLVCLISDFYPGAVTVAWKADSSPVKAGVETTTPSKQSNNKYAASSYLSLTPEQWKSHRSYSCQVTHEGSTVEKTVAPTECS

SEQ ID NO: 60 - protein, 11 aa, Artificial Sequence
  Description of Artificial Sequence: Synthetic peptide
QVWDSSSDHVA

SEQ ID NO: 61 - protein, 109 aa, Artificial Sequence
  Description of Artificial Sequence: Synthetic polypeptide
SYVLTQPPSVSVAPGQTARITCGGNNIGSKNVYWYQQKPGQAPVLVVHDDSDRPSGIPERFSGSNSGNTATLTISRVEVGDEADYSCQVWDSSSDHVAFGGGTKLTVLG

SEQ ID NO: 62 - protein, 214 aa, Artificial Sequence
  Description of Artificial Sequence: Synthetic polypeptide
SYVLTQPPSVSVAPGQTARITCGGNNIGSKNVYWYQQKPGQAPVLVVHDDSDRPSGIPERFSGSNSGNTATLTISRVEVGDEADYSCQVWDSSSDHVAFGGGTKLTVLGQPKAAPSVTLFPPSSEELQANKATLVCLISDFYPGAVTVAWKADSSPVKAGVETTTPSKQSNNKYAASSYLSLTPEQWKSHRSYSCQVTHEGSTVEKTVAPTECS

SEQ ID NO: 63 - protein, 11 aa, Artificial Sequence
  Description of Artificial Sequence: Synthetic peptide
QVWDSSSDHVW

SEQ ID NO: 64 - protein, 109 aa, Artificial Sequence
  Description of Artificial Sequence: Synthetic polypeptide
SYVLTQPPSVSVAPGQTARITCGGNNIGSKNVYWYQQKPGQAPVLVVHDDSDRPSGIPERFSGSNSGNTATLTISRVEVGDEADYSCQVWDSSSDHVWFGGGTKLTVLG

SEQ ID NO: 65 - protein, 214 aa, Artificial Sequence
  Description of Artificial Sequence: Synthetic polypeptide
SYVLTQPPSVSVAPGQTARITCGGNNIGSKNVYWYQQKPGQAPVLVVHDDSDRPSGIPERFSGSNSGNTATLTISRVEVGDEADYSCQVWDSSSDHVWFGGGTKLTVLGQPKAAPSVTLFPPSSEELQANKATLVCLISDFYPGAVTVAWKADSSPVKAGVETTTPSKQSNNKYAASSYLSLTPEQWKSHRSYSCQVTHEGSTVEKTVAPTECS

SEQ ID NO: 66 - protein, 11 aa, Artificial Sequence
  Description of Artificial Sequence: Synthetic peptide
GGNNIDSKNVY

SEQ ID NO: 67 - protein, 109 aa, Artificial Sequence
  Description of Artificial Sequence: Synthetic polypeptide
SYVLTQPPSVSVAPGQTARITCGGNNIDSKNVYWYQQKPGQAPVLVVHDDSDRPSGIPERFSGSNSGNTATLTISRVEVGDEADYSCQVWDSSSDHVVFGGGTKLTVLG

SEQ ID NO: 68 - protein, 214 aa, Artificial Sequence
  Description of Artificial Sequence: Synthetic polypeptide
SYVLTQPPSVSVAPGQTARITCGGNNIDSKNVYWYQQKPGQAPVLVVHDDSDRPSGIPERFSGSNSGNTATLTISRVEVGDEADYSCQVWDSSSDHVVFGGGTKLTVLGQPKAAPSVTLFPPSSEELQANKATLVCLISDFYPGAVTVAWKADSSPVKAGVETTTPSKQSNNKYAASSYLSLTPEQWKSHRSYSCQVTHEGSTVEKTVAPTECS

SEQ ID NO: 69 - DNA, 351 bp, Artificial Sequence
  Description of Artificial Sequence: Synthetic polynucleotide
caggtgcagctgcaggaatctggccctggcctggtcaagcccagccagaccctgagcctgacctgtaccgtgtccggcggcagcatcagcaacggcggctactactggtcctggatcagacagcaccccggcaagggcctggaatggatcggctacatctactacagcggcagcacctactacaaccccagcctgaagtccagagtgaccatcagcgtggacaccagcaagaaccagttcagcctgaagctgagcagcgtgacagccgccgacaccgccgtgtactactgcgccagcctgggcaattggttcgactactggggccagggcaccctcgtgacagtgtcctca

SEQ ID NO: 70 - DNA, 978 bp, Artificial Sequence
  Description of Artificial Sequence: Synthetic polynucleotide
gctagcaccaagggccccagcgtgttccccctggccccttgtagcagaagcaccagcgagagcacagccgccctgggctgcctggtgaaagactacttccccgagcccgtcaccgtgtcctggaacagcggagccctgaccagcggcgtgcacacctttccagccgtgctgcagagcagcggcctgtacagcctgagcagcgtggtgacagtgccctccagcagcctgggcaccaagacctacacctgtaacgtggaccacaagcccagcaacaccaaggtggacaagcgggtggaatctaagtacggcccaccctgccccccctgccctgcccctgaatttctgggcggaccctccgtgttcctgttccccccaaagcccaaggacaccctgtatatcactcgggagcccgaagtgacctgcgtggtggtggacgtgtcccaggaagatcccgaggtccagttcaattggtacgtggacggcgtggaagtgcacaacgccaagaccaagcccagagaggaacagttcaacagcacctaccgggtggtgtccgtgctgaccgtgctgcaccaggactggctgaacggcaaagagtacaagtgcaaagtctccaacaagggcctgcccagctccatcgagaaaaccatcagcaaggccaagggccagccccgcgagcctcaggtgtacacactgccccccagccaggaagagatgaccaagaaccaggtgtccctgacctgtctggtgaaaggcttctaccccagcgatatcgccgtggaatgggagagcaacggccagcccgagaacaactacaagaccaccccccctgtgctggacagcgacggcagcttcttcctgtactcccggctgaccgtggacaagagccggtggcaggaaggcaacgtcttcagctgcagcgtgatgcacgaggccctgcacaaccactacacccagaagtccctgagcctgagcctgggc

SEQ ID NO: 71 - DNA, 327 bp, Artificial Sequence
  Description of Artificial Sequence: Synthetic polynucleotide
agctacgtgctgacccagcctcctagcgtgtccgtggcccctggccagaccgccagaatcacctgtggcggcaacaacatcggcagcaagaacgtgtactggtatcagcagaagcccggccaggcccccgtgctggtggtgcacgacgacagcgacagacccagcggcatccccgagcggttcagcggcagcaacagcggcaataccgccaccctgaccatcagccgggtggaagtgggcgacgaggccgactacagctgccaggtctgggacagcagcagcgaccacgtggtgttcggcggaggcaccaagctgaccgtcctaggt

SEQ ID NO: 72 - DNA, 315 bp, Artificial Sequence
  Description of Artificial Sequence: Synthetic polynucleotide
cagcccaaggccgctcccagcgtgaccctgttccccccaagcagcgaggaactgcaggccaacaaggccaccctggtgtgcctgatcagcgacttctaccctggggccgtgaccgtggcctggaaggccgatagcagccctgtgaaggccggcgtggaaaccaccaccccctccaagcagagcaacaacaaatacgccgccagcagctacctgtccctgacccccgagcagtggaagtcccaccggtcctacagctgccaggtgacacacgagggcagcaccgtggaaaagaccgtggcccccaccgagtgcagc

SEQ ID NO: 73 - protein, 117 aa, Artificial Sequence
  Description of Artificial Sequence: Synthetic polypeptide
  MOD_RES (26)..(26): Gly, Ala, Ser, Leu, Tyr, Asp, Gln, Lys, His or Trp
  MOD_RES (27)..(27): Gly, Ala, Ser, Leu, Tyr, Asp, Gln, Lys, His or Trp
  MOD_RES (28)..(28): Ser, Ala, Leu, Tyr, Asp, Gln, Lys, His or Trp
  MOD_RES (29)..(29): Ile, Ala, Ser, Leu, Tyr, Asp, Gln, Lys, His or Trp
  MOD_RES (30)..(30): Ser, Ala, Leu, Tyr, Asp, Gln, Lys, His or Trp
  MOD_RES (31)..(31): Asn, Ala, Ser, Leu, Tyr, Asp, Gln, Lys, His or Trp
  MOD_RES (32)..(32): Gly, Ala, Ser, Leu, Tyr, Asp, Gln, Lys, His or Trp
  MOD_RES (33)..(33): Gly, Ala, Ser, Leu, Tyr, Asp, Gln, Lys, His or Trp
  MOD_RES (34)..(34): Tyr, Ala, Ser, Leu, Asp, Gln, Lys, His or Trp
  MOD_RES (35)..(35): Tyr, Ala, Ser, Leu, Asp, Gln, Lys, His or Trp
  MOD_RES (36)..(36): Trp, Ala, Ser, Leu, Tyr, Asp, Gln, Lys or His
  MOD_RES (37)..(37): Ser, Ala, Leu, Tyr, Asp, Gln, Lys, His or Trp
  MOD_RES (52)..(52): Tyr, Ala, Ser, Leu, Asp, Gln, Lys, His or Trp
  MOD_RES (53)..(53): Ile, Ala, Ser, Leu, Tyr, Asp, Gln, Lys, His or Trp
  MOD_RES (54)..(54): Tyr, Ala, Ser, Leu, Asp, Gln, Lys, His or Trp
  MOD_RES (55)..(55): Tyr, Ala, Ser, Leu, Asp, Gln, Lys, His or Trp
  MOD_RES (56)..(56): Ser, Ala, Leu, Asp, Gln, Lys, His or Trp
  MOD_RES (57)..(57): Gly, Ala, Ser, Leu, Tyr, Asp, Gln, Lys, His or Trp
  MOD_RES (58)..(58): Ser, Ala, Leu, Tyr, Asp, Gln, Lys, His or Trp
  MOD_RES (59)..(59): Thr, Ala, Ser, Leu, Tyr, Asp, Gln, Lys, His or Trp
  MOD_RES (60)..(60): Tyr, Ala, Ser, Leu, Asp, Gln, Lys, His or Trp
  MOD_RES (98)..(98): Ala, Ser, Leu, Tyr, Asp, Gln, Lys, His, Trp or Pro
  MOD_RES (99)..(99): Ser, Ala, Leu, Tyr, Asp, Gln, Lys, His, Trp or Pro
  MOD_RES (100)..(100): Leu, Ala, Ser, Tyr, Asp, Gln, Lys, His, Trp or Pro
  MOD_RES (101)..(101): Gly, Ala, Ser, Leu, Tyr, Asp, Gln, Lys, His, Trp or Pro
  MOD_RES (102)..(102): Asn, Ala, Ser, Leu, Tyr, Asp, Gln, Lys, His, Trp or Pro
  MOD_RES (103)..(103): Trp, Ala, Ser, Leu, Tyr, Asp, Gln, Lys, His or Pro
  MOD_RES (104)..(104): Phe, Ala, Ser, Leu, Tyr, Asp, Gln, Lys, His, Trp or Pro
  MOD_RES (105)..(105): Asp, Ala, Ser, Leu, Tyr, Gln, Lys, His, Trp or Pro
  MOD_RES (106)..(106): Tyr, Ala, Ser, Leu, Asp, Gln, Lys, His, Trp or Pro
QVQLQESGPGLVKPSQTLSLTCTVSXXXXXXXXXXXXWIRQHPGKGLEWIGXXXXXXXXXYNPSLKSRVTISVDTSKNQFSLKLSSVTAADTAVYYCXXXXXXXXXWGQGTLVTVSS

SEQ ID NO: 74 - protein, 109 aa, Artificial Sequence
  Description of Artificial Sequence: Synthetic polypeptide
  MOD_RES (23)..(23): Gly, Ala, Ser, Leu, Tyr, Asp, Gln, Lys, His or Trp
  MOD_RES (24)..(24): Gly, Ala, Ser, Leu, Tyr, Asp, Gln, Lys, His or Trp
  MOD_RES (25)..(25): Asn, Ala, Ser, Leu, Tyr, Asp, Gln, Lys, His or Trp
  MOD_RES (26)..(26): Asn, Ala, Ser, Leu, Tyr, Asp, Gln, Lys, His or Trp
  MOD_RES (27)..(27): Ile, Ala, Ser, Leu, Tyr, Asp, Gln, Lys, His or Trp
  MOD_RES (28)..(28): Gly, Ala, Ser, Leu, Tyr, Asp, Gln, Lys, His or Trp
  MOD_RES (29)..(29): Ser, Ala, Leu, Tyr, Asp, Gln, Lys, His or Trp
  MOD_RES (30)..(30): Lys, Ala, Ser, Leu, Tyr, Asp, Gln, His or Trp
  MOD_RES (31)..(31): Asn, Ala, Ser, Leu, Tyr, Asp, Gln, Lys, His or Trp
  MOD_RES (32)..(32): Val, Ala, Ser, Leu, Tyr, Asp, Gln, Lys, His or Trp
  MOD_RES (33)..(33): Tyr, Ala, Ser, Leu, Asp, Gln, Lys, His or Trp
  MOD_RES (49)..(49): Asp, Ala, Ser, Leu, Tyr, Gln, Lys, His or Trp
  MOD_RES (50)..(50): Asp, Ala, Ser, Leu, Tyr, Gln, Lys, His or Trp
  MOD_RES (51)..(51): Ser, Ala, Leu, Tyr, Asp, Gln, Lys, His or Trp
  MOD_RES (52)..(52): Asp, Ala, Ser, Leu, Tyr, Gln, Lys, His or Trp
  MOD_RES (53)..(53): Arg, Ala, Ser, Leu, Tyr, Asp, Gln, Lys, His or Trp
  MOD_RES (54)..(54): Pro, Ala, Ser, Leu, Tyr, Asp, Gln, Lys, His or Trp
  MOD_RES (55)..(55): Ser, Ala, Leu, Tyr, Asp, Gln, Lys, His or Trp
  MOD_RES (88)..(88): Gln, Ala, Ser, Leu, Tyr, Asp, Lys, His, Trp or Pro
  MOD_RES (89)..(89): Val, Ala, Ser, Leu, Tyr, Asp, Gln, Lys, His, Trp or Pro
  MOD_RES (90)..(90): Trp, Ala, Ser, Leu, Tyr, Asp, Gln, Lys, His or Pro
  MOD_RES (91)..(91): Asp, Ala, Ser, Leu, Tyr, Gln, Lys, His, Trp or Pro
  MOD_RES (92)..(92): Ser, Ala, Leu, Tyr, Asp, Gln, Lys, His, Trp or Pro
  MOD_RES (93)..(93): Ser, Ala, Leu, Tyr, Asp, Gln, Lys, His, Trp or Pro
  MOD_RES (94)..(94): Ser, Ala, Leu, Tyr, Asp, Gln, Lys, His, Trp or Pro
  MOD_RES (95)..(95): Asp, Ala, Ser, Leu, Tyr, Gln, Lys, His, Trp or Pro
  MOD_RES (96)..(96): His, Ala, Ser, Leu, Tyr, Asp, Gln, Lys, Trp or Pro
  MOD_RES (97)..(97): Val, Ala, Ser, Leu, Tyr, Asp, Gln, Lys, His, Trp or Pro
  MOD_RES (98)..(98): Val, Ala, Ser, Leu, Tyr, Asp, Gln, Lys, His, Trp or Pro
SYVLTQPPSVSVAPGQTARITCXXXXXXXXXXXWYQQKPGQAPVLVVHXXXXXXXGIPERFSGSNSGNTATLTISRVEVGDEADYSCXXXXXXXXXXXFGGGTKLTVLG

SEQ ID NO: 75 - protein, 109 aa, Artificial Sequence
  Description of Artificial Sequence: Synthetic polypeptide
  MOD_RES (24)..(24): Gly or Lys
  MOD_RES (25)..(25): Asn or Asp
  MOD_RES (26)..(26): Asn or His
  MOD_RES (27)..(27): Ile or Ala
  MOD_RES (28)..(28): Gly or Asp
  MOD_RES (29)..(29): Ser or Lys
  MOD_RES (31)..(31): Asn or His
  MOD_RES (32)..(32): Val or Ala
  MOD_RES (51)..(51): Ser or Leu
  MOD_RES (52)..(52): Asp or Ser
  MOD_RES (91)..(91): Asp or Leu
  MOD_RES (96)..(96): His, Ser, Tyr or Asp
  MOD_RES (98)..(98): Val, Ala or Trp
SYVLTQPPSVSVAPGQTARITCGXXXXXXKXXYWYQQKPGQAPVLVVHDDXXRPSGIPERFSGSNSGNTATLTISRVEVGDEADYSCQVWXSSSDXVXFGGGTKLTVLG